European Patent Application EP 4 729 544 A1, published April 22, 2026. Title: 소세포폐암 진단 및 치료를 위한 타겟으로서 클라우딘-3의 용도. Applicant: 에이비온 주식회사. The sequence listing filed with the application follows.

SEQUENCE LISTING (8 sequences)

SEQ ID NO: 1 - protein, 5 aa, synthetic construct
SYAMS

SEQ ID NO: 2 - protein, 16 aa, synthetic construct
IINPSGASTSHAQRFQ

SEQ ID NO: 3 - protein, 10 aa, synthetic construct
RYGRYGSFDI

SEQ ID NO: 4 - protein, 13 aa, synthetic construct
SGSTSNIGRNYVS

SEQ ID NO: 5 - protein, 7 aa, synthetic construct
DTSNKHF

SEQ ID NO: 6 - protein, 9 aa, synthetic construct
QSYDSSKVV

SEQ ID NO: 7 - protein, 448 aa, synthetic construct
EVQLLESGGGLVQPGGSLRLSCAASGFTFSSYAMSWVRQAPGKGLEWVSIINPSGASTSHAQRFQGRFTISRDNSKNTLYLQMNSLRAEDTAVYYCARYGRYGSFDIWGQGTLVTVSSASTKGPSVFPLAPSSKSTSGGTAALGCLVKDYFPEPVTVSWNSGALTSGVHTFPAVLQSSGLYSLSSVVTVPSSSLGTQTYICNVNHKPSNTKVDKKVEPKSCDKTHTCPPCPAPELLGGPSVFLFPPKPKDTLMISRTPEVTCVVVDVSHEDPEVKFNWYVDGVEVHNAKTKPREEQYNSTYRVVSVLTVLHQDWLNGKEYKCKVSNKALPAPIEKTISKAKGQPREPQVYTLPPSRDELTKNQVSLTCLVKGFYPSDIAVEWESNGQPENNYKTTPPVLDSDGSFFLYSKLTVDKSRWQQGNVFSCSVMHEALHNHYTQKSLSLSPGK

SEQ ID NO: 8 - protein, 215 aa, synthetic construct
QSVLTQPPSASGTPGQRVTISCSGSTSNIGRNYVSWYQQLPGTAPKLLIYDTSNKHFGVPDRFSGSKSGTSASLAISGLRSEDEADYYCQSYDSSKVVFGGGTKLTVLRTVAAPSVFIFPPSDEQLKSGTASVVCLLNNFYPREAKVQWKVDNALQSGNSQESVTEQDSKDSTYSLSSTLTLSKADYEKHKVYACEVTHQGLSSPVTKSFNRGEC